European Patent Application EP 4 603 499 A1, published August 20, 2025. Title: Peptide Having Activity of Promoting Hair Growth and Inhibiting Hair Loss and Uses Thereof. Applicant: CAREGENE CO., LTD. Application KR. The sequence listing filed with the application follows.

SEQUENCE LISTING (23 sequences)

SEQ ID NO: 1 - protein, 7 aa, synthetic construct
RHVLKRR

SEQ ID NO: 2 - DNA, 20 bp, synthetic construct
  source 1..20: mol_type = other DNA
ccagctattgtaacacctca

SEQ ID NO: 3 - DNA, 20 bp, synthetic construct
  source 1..20: mol_type = other DNA
ttcagatgtaggcagctgtc

SEQ ID NO: 4 - DNA, 25 bp, synthetic construct
  source 1..25: mol_type = other DNA
accagcagcgactctgaggaggaac

SEQ ID NO: 5 - DNA, 26 bp, synthetic construct
  source 1..26: mol_type = other DNA
tgaccctcttggcagcaggatagtcc

SEQ ID NO: 6 - DNA, 28 bp, synthetic construct
  source 1..28: mol_type = other DNA
accttcgttgccctctgtgccacagatg

SEQ ID NO: 7 - DNA, 21 bp, synthetic construct
  source 1..21: mol_type = other DNA
aggcccggaggcagtccgggt

SEQ ID NO: 8 - DNA, 20 bp, synthetic construct
  source 1..20: mol_type = other DNA
ggagccaaaagggtcatcat

SEQ ID NO: 9 - DNA, 20 bp, synthetic construct
  source 1..20: mol_type = other DNA
gtgatggcatggactgtggt

SEQ ID NO: 10 - DNA, 20 bp, synthetic construct
  source 1..20: mol_type = other DNA
gatcatcgagctgagacgca

SEQ ID NO: 11 - DNA, 20 bp, synthetic construct
  source 1..20: mol_type = other DNA
ctggccccagggtatctagt

SEQ ID NO: 12 - DNA, 20 bp, synthetic construct
  source 1..20: mol_type = other DNA
ccctcaaggatgccaggaac

SEQ ID NO: 13 - DNA, 19 bp, synthetic construct
  source 1..19: mol_type = other DNA
cactgctacctccggcaag

SEQ ID NO: 14 - DNA, 20 bp, synthetic construct
  source 1..20: mol_type = other DNA
ccaaatccgcaccaaggtca

SEQ ID NO: 15 - DNA, 21 bp, synthetic construct
  source 1..21: mol_type = other DNA
gtattgattgccaggaggggg

SEQ ID NO: 16 - DNA, 20 bp, synthetic construct
  source 1..20: mol_type = other DNA
cgcggcgtatccgtgtcctc

SEQ ID NO: 17 - DNA, 24 bp, synthetic construct
  source 1..24: mol_type = other DNA
agcctgttccgtctcaaacttggt

SEQ ID NO: 18 - DNA, 20 bp, synthetic construct
  source 1..20: mol_type = other DNA
cggtcaagtcggaaaattca

SEQ ID NO: 19 - DNA, 20 bp, synthetic construct
  source 1..20: mol_type = other DNA
gaggagctgggatgtggtaa

SEQ ID NO: 20 - DNA, 20 bp, synthetic construct
  source 1..20: mol_type = other DNA
gccgtctatacggacatgcc

SEQ ID NO: 21 - DNA, 20 bp, synthetic construct
  source 1..20: mol_type = other DNA
gcagtacacctgactgtccc

SEQ ID NO: 22 - DNA, 20 bp, synthetic construct
  source 1..20: mol_type = other DNA
caggactgggtgatggtgtc

SEQ ID NO: 23 - DNA, 20 bp, synthetic construct
  source 1..20: mol_type = other DNA
tctgagggtgagagcctgaa